European Patent Specification EP 3 812 402 B1, published November 20, 2024. Title: BIFUNCTIONAL ANGIOGENESIS INHIBITOR AND USE THEREOF. Applicant: RemeGen Co., Ltd. The sequence listing filed with the application follows.

SEQUENCE LISTING (3 sequences)

SEQ ID NO: 1 - protein, 641 aa, Unknown
GRPFVEMYSEIPEIIHMTEGRELVIPCRVTSPNITVTLKKFPLDTLIPDGKRIIWDSRKGFIISNATYKEIGLLTCEATVNGHLYKTNYLTHRQTNTIIDVVLSPSHGIELSVGEKLVLNCTARTELNVGIDFNWEYPSSKHQHKKLVNRDLKTQSGSEMKKFLSTLTIDGVTRSDQGLYTCAASSGLMTKKNSTFVRVHEKPVAPYWTSPEKMEKKLHAVPAAKTVKFKCPSSGTPNPTLRWLKNGKEFKPDHRIGGYKVRYATWSIIMDSVVPSDKGNYTCIVENEYGSINHTYQLDVVERSPHRPILQAGLPANKTVALGSNVEFMCKVYSDPQPHIQWLKHIEVNGSKIGPDNLPYVQILKTAGVNTTDKEMEVLHLRNVSFEDAGEYTCLAGNSIGLSHHSAWLTVLEADKTHTCPPCPAPELLGGPSVFLFPPKPKDTLMISRTPEVTCVVVDVSHEDPEVKFNWYVDGVEVHNAKTKPREEQYNSTYRVVSVLTVLHQDWLNGKEYKCKVSNKALPAPIEKTISKAKGQPREPQVYTLPPSRDELTKNQVSLTCLVKGFYPSDIAVEWESNGQPENNYKTTPPVLDSDGSFFLYSKLTVDKSRWQQGNVFSCSVMHEALHNHYTQKSLSLSPGK

SEQ ID NO: 2 - protein, 658 aa, Unknown
GRPFVEMYSEIPEIIHMTEGRELVIPCRVTSPNITVTLKKFPLDTLIPDGKRIIWDSRKGFIISNATYKEIGLLTCEATVNGHLYKTNYLTHRQTNTIIDVVLSPSHGIELSVGEKLVLNCTARTELNVGIDFNWEYPSSKHQHKKLVNRDLKTQSGSEMKKFLSTLTIDGVTRSDQGLYTCAASSGLMTKKNSTFVRVHEKPNPVAPYWTSPEKMEKKLHAVPAAKTVKFKCPSSGTPNPTLRWLKNGKEFKPDHRIGGYKVRYATWSIIMDSVVPSDKGNYTCIVENEYGSINHTYQLDVVERSPHRPILQAGLPANKTVALGSNVEFMCKVYSDPQPHIQWLKHIEVNGSKIGPDNLPYVQILKTAGVNTTDKEMEVLHLRNVSFEDAGEYTCLAGNSIGLSHHSAWLTVLEALEERPAVMTSPLYLEDKTHTCPPCPAPELLGGPSVFLFPPKPKDTLMISRTPEVTCVVVDVSHEDPEVKFNWYVDGVEVHNAKTKPREEQYNSTYRVVSVLTVLHQDWLNGKEYKCKVSNKALPAPIEKTISKAKGQPREPQVYTLPPSRDELTKNQVSLTCLVKGFYPSDIAVEWESNGQPENNYKTTPPVLDSDGSFFLYSKLTVDKSRWQQGNVFSCSVMHEALHNHYTQKSLSLSPGK

SEQ ID NO: 3 - DNA, 1923 bp, Unknown
ggtagaccattcgtagagatgtacagtgaaatccccgaaattatacacatgactgaaggaagggagctcgtcattccctgccgggttacgtcacctaacatcactgttactttaaaaaagtttccacttgacactttgatccctgatggaaaacgcataatctgggacagtagaaagggcttcatcatatcaaatgcaacgtacaaagaaatagggcttctgacctgtgaagcaacagtcaatgggcatttgtataagacaaactatctcacacatcgacaaaccaatacaatcatagatgtggttctgagtccgtctcatggaattgaactatctgttggagaaaagcttgtcttaaattgtacagcaagaactgaactaaatgtggggattgacttcaactgggaatacccttcttcgaagcatcagcataagaaacttgtaaaccgagacctaaaaacccagtctgggagtgagatgaagaaatttttgagcaccttaactatagatggtgtaacccggagtgaccaaggattgtacacctgtgcagcatccagtgggctgatgaccaagaagaacagcacatttgtcagggtccatgaaaaacccgtagctccatattggacatccccagaaaagatggaaaagaaattgcatgcagtgccggctgccaagacagtgaagttcaaatgcccttccagtgggaccccaaaccccacactgcgctggttgaaaaatggcaaagaattcaaacctgaccacagaattggaggctacaaggtccgttatgccacctggagcatcataatggactctgtggtgccctctgacaagggcaactacacctgcattgtggagaatgagtacggcagcatcaaccacacataccagctggatgtcgtggagcggtcccctcaccggcccatcctgcaagcagggttgcccgccaacaaaacagtggccctgggtagcaacgtggagttcatgtgtaaggtgtacagtgacccgcagccgcacatccagtggctaaagcacatcgaggtgaatgggagcaagattggcccagacaacctgccttatgtccagatcttgaagactgctggagttaataccaccgacaaagagatggaggtgcttcacttaagaaatgtctcctttgaggacgcaggggagtatacgtgcttggcgggtaactctatcggactctcccatcactctgcatggttgaccgttctggaagccgacaaaactcacacatgcccaccgtgcccagcacctgaactcctggggggaccgtcagtcttcctcttccccccaaaacccaaggacaccctcatgatctcccggacccctgaggtcacatgcgtggtggtggacgtgagccacgaagaccctgaggtcaagttcaactggtacgtggacggcgtggaggtgcataatgccaagacaaagccgcgggaggagcagtacaacagcacgtaccgtgtggtcagcgtcctcaccgtcctgcaccaggactggctgaatggcaaggagtacaagtgcaaggtctccaacaaagccctcccagcccccatcgagaaaaccatctccaaagccaaagggcagccccgagaaccacaggtgtacaccctgcccccatcccgggatgagctgaccaagaaccaggtcagcctgacctgcctggtcaaaggcttctatcccagcgacatcgccgtggagtgggagagcaatgggcagccggagaacaactacaagaccacgcctcccgtgctggactccgacggctccttcttcctctacagcaagctcaccgtggacaagagcaggtggcagcaggggaacgtcttctcatgctccgtgatgcatgaggctctgcacaaccactacacgcagaagagcctctccctgtctccgggtaaa